European Patent Application EP 4 541 906 A1, published April 23, 2025. Title: Primers, and method and kit for detecting DNA. Applicant: Hitachi High-Tech Corporation. The sequence listing filed with the application follows.

SEQUENCE LISTING (7 sequences)

SEQ ID NO: 1 - DNA, 29 bp, Artificial
  synthetic polynucleotide
gtcacattttcattatttttattataagg

SEQ ID NO: 2 - DNA, 22 bp, Artificial
  synthetic polynucleotide
gtatcgtcaaggcactcttgcc

SEQ ID NO: 3 - DNA, 16 bp, Artificial
  synthetic polynucleotide
ttggagctggtggcgt

SEQ ID NO: 4 - DNA, 15 bp, Artificial
  synthetic polynucleotide
ctggtgacgtaggca

SEQ ID NO: 5 - DNA, 103 bp, Artificial
  synthetic polynucleotide
gtcacattttcattatttttattataaggcctgctgaaaatgactgaatataaacttgtggtagttggagctggtgacgtaggcaagagtgccttgacgatac

SEQ ID NO: 6 - DNA, 103 bp, Artificial
  synthetic polynucleotide
gtcacattttcattatttttattataaggcctgctgaaaatgactgaatataaacttgtggtagttggagctggtgacgtaggcaagagtgaattgacgatac

SEQ ID NO: 7 - DNA, 109 bp, Artificial
  synthetic polynucleotide
gtcacattttcattatttttattataaggcctgctgaaaatgactgaatataaacttgtggtagttggagctggtgacgtaggcaagagtgaattgacgataccgtcaa